European Patent Application EP 4 582 456 A1, published July 9, 2025. Title: ENHANCED RECEPTOR, AND IMMUNE CELL EXPRESSING ENHANCED RECEPTOR AND USE THEREOF. Applicant: Chineo Medical Technology Co., Ltd. Application EP. The sequence listing filed with the application follows.

SEQUENCE LISTING (22 sequences)

SEQ ID NO: 1 - DNA, 423 bp, Homo sapiens
  source 1..423: mol_type = genomic DNA
atgcggtggtgcctgctgctgatctgggcccaggggctgaggcaggcccccctggccagcggcatgatgacaggcacaattgagacaacaggcaacatcagcgccgagaagggcgggagcatcatcctgcagtgccacctgagcagcaccaccgcccaggtgacacaggtgaactgggagcagcaggaccagctgctggccatctgcaacgccgatctgggctggcacatcagcccaagcttcaaggatagggtggcccccggccccggcctggggctgaccctgcagagcctgaccgtcaacgacaccggggagtacttctgcatctaccacacataccccgacggcacctacaccgggcggatcttcctggaggtgctggagagcagcgtggccgagcacggcgccagattccagatcccc

SEQ ID NO: 2 - DNA, 111 bp, Homo sapiens
  source 1..111: mol_type = genomic DNA
aggcgggatcagcggctgccccccgacgcccacaagccccccggcgggggctccttcaggacacccatccaggaggagcaggccgatgcccacagcaccctggccaagatc

SEQ ID NO: 3 - DNA, 78 bp, Homo sapiens
  source 1..78: mol_type = genomic DNA
gtggccgccatcctcgggctggggctggtcctggggctgctgggccccctggccatcctgctggccctgtacctgctg

SEQ ID NO: 4 - DNA, 465 bp, synthetic construct
  source 1..465: mol_type = other DNA
atgcagatcccacaggcgccctggccagtcgtctgggcggtgctacaactgggctggcggccaggatggttcttagactccccagacaggccctggaacccccccaccttctccccagccctgctcgtggtgaccgaaggggacaacgccaccttcacctgcagcttctccaacacatcggagagcttcgtgctaaactggtaccgcatgagccccagcaaccagacggacaagctggccgccttccccgaggaccgtattaataggagtcaggactgccgcttccgtgtcacacaactgcccaacgggcgtgacttccacatgagcgtggtcagggcccggcgcaatgacagcggcacctacctctgtggggccatctccctgtctactccggtgtggatcaaagagagcctgcgggcagagctcagggtgacagagagaagggcagaagtgcccacagcccac

SEQ ID NO: 5 - DNA, 123 bp, Homo sapiens
  source 1..123: mol_type = genomic DNA
aggagtaagaggagcaggctcctgcacagtgactacatgaacatgactccccgccgccccgggcccacccgcaagcattaccagccctatgccccaccacgcgacttcgcagcctatcgctcc

SEQ ID NO: 6 - DNA, 117 bp, Homo sapiens
  source 1..117: mol_type = genomic DNA
tgtccaagtcccctatttcccggaccttctaagcccttttgggtgctggtggtggttggtggagtcctggcttgctatagcttgctagtaacagtggcctttattattttctgggtg

SEQ ID NO: 7 - DNA, 783 bp, synthetic construct
  source 1..783: mol_type = other DNA
atggccttaccagtgaccgccttgctcctgccgctggccttgctgctccacgccgccaggccggacatccagatgacccagagccctagcagcctgagcgctagcgtgggagatagagtgaccatcacctgcagggcctctcaggatgtgtctacagccgtggcttggtaccagcagaagccaggaaaggcccccaagctgctgatctacagcgcctctttcctgtacagcggcgtgcctagcagattcagcggcagcggaagcggcaccgatttcaccctgaccatcagcagcctgcagccagaggacttcgccacctactactgccagcagtacctgtaccacccagccaccttcggacagggcaccaaggtggagatcaagggtggcggtggctcgggcggtggtgggtcgggtggcggcggatctgaggtgcagctggtggaatcaggaggaggactggtgcagccaggaggatctctgagactgtcttgcgccgccagcggctttacattcagcgactcttggatccattgggtgcgccaggctccaggaaaaggactcgagtgggtggcttggatcagcccttacggcggcagcacctactacgccgatagcgtgaagggcaggttcaccatcagcgccgataccagcaagaacaccgcctacctgcagatgaacagcctgagggccgaggataccgccgtgtactattgcgccaggaggcattggccaggcggatttgactattggggccagggaacactggtgaccgtgtccagc

SEQ ID NO: 8 - DNA, 465 bp, Homo sapiens
  source 1..465: mol_type = genomic DNA
atgcagatcccacaggcgccctggccagtcgtctgggcggtgctacaactgggctggcggccaggatggttcttagactccccagacaggccctggaacccccccaccttctccccagccctgctcgtggtgaccgaaggggacaacgccaccttcacctgcagcttctccaacacatcggagagcttcgtgctaaactggtaccgcatgagccccagcaaccagacggacaagctggccgccttccccgaggaccgcagccagcccggccaggactgccgcttccgtgtcacacaactgcccaacgggcgtgacttccacatgagcgtggtcagggcccggcgcaatgacagcggcacctacctctgtggggccatctccctggcccccaaggcgcagatcaaagagagcctgcgggcagagctcagggtgacagagagaagggcagaagtgcccacagcccac

SEQ ID NO: 9 - protein, 141 aa, Homo sapiens
MRWCLLLIWAQGLRQAPLASGMMTGTIETTGNISAEKGGSIILQCHLSSTTAQVTQVNWEQQDQLLAICNADLGWHISPSFKDRVAPGPGLGLTLQSLTVNDTGEYFCIYHTYPDGTYTGRIFLEVLESSVAEHGARFQIP

SEQ ID NO: 10 - protein, 37 aa, Homo sapiens
RRDQRLPPDAHKPPGGGSFRTPIQEEQADAHSTLAKI

SEQ ID NO: 11 - protein, 26 aa, Homo sapiens
VAAILGLGLVLGLLGPLAILLALYLL

SEQ ID NO: 12 - protein, 155 aa, synthetic construct
MQIPQAPWPVVWAVLQLGWRPGWFLDSPDRPWNPPTFSPALLVVTEGDNATFTCSFSNTSESFVLNWYRMSPSNQTDKLAAFPEDRINRSQDCRFRVTQLPNGRDFHMSVVRARRNDSGTYLCGAISLSTPVWIKESLRAELRVTERRAEVPTAH

SEQ ID NO: 13 - protein, 41 aa, Homo sapiens
RSKRSRLLHSDYMNMTPRRPGPTRKHYQPYAPPRDFAAYRS

SEQ ID NO: 14 - protein, 39 aa, Homo sapiens
CPSPLFPGPSKPFWVLVVVGGVLACYSLLVTVAFIIFWV

SEQ ID NO: 15 - protein, 261 aa, synthetic construct
MALPVTALLLPLALLLHAARPDIQMTQSPSSLSASVGDRVTITCRASQDVSTAVAWYQQKPGKAPKLLIYSASFLYSGVPSRFSGSGSGTDFTLTISSLQPEDFATYYCQQYLYHPATFGQGTKVEIKGGGGSGGGGSGGGGSEVQLVESGGGLVQPGGSLRLSCAASGFTFSDSWIHWVRQAPGKGLEWVAWISPYGGSTYYADSVKGRFTISADTSKNTAYLQMNSLRAEDTAVYYCARRHWPGGFDYWGQGTLVTVSS

SEQ ID NO: 16 - protein, 155 aa, Homo sapiens
MQIPQAPWPVVWAVLQLGWRPGWFLDSPDRPWNPPTFSPALLVVTEGDNATFTCSFSNTSESFVLNWYRMSPSNQTDKLAAFPEDRSQPGQDCRFRVTQLPNGRDFHMSVVRARRNDSGTYLCGAISLAPKAQIKESLRAELRVTERRAEVPTAH

SEQ ID NO: 17 - protein, 603 aa, synthetic construct
METLLGLLILWLQLQWVSSKQEVTQIPAALSVPEGENLVLNCSFTDSAIYNLQWFRQDPGKGLTSLLLIQSSQREQTSGRLNASLDKSSGRSTLYIAASQPGDSATYLCAVRPLYGGSYIPTFGRGTSLIVHPYIQNPDPAVYQLRDSKSSDKSVCLFTDFDSQTNVSQSKDSDVYITDKTVLDMRSMDFKSNSAVAWSNKSDFACANAFNNSIIPEDTFFPSPESSCDVKLVEKSFETDTNLNFQNLSVIGFRILLLKVAGFNLLMTLRLWSSQCTNYALLKLAGDVESNPGPMSIGLLCCAALSLLWAGPVNAGVTQTPKFQVLKTGQSMTLQCAQDMNHEYMSWYRQDPGMGLRLIHYSVGAGITDQGEVPNGYNVSRSTTEDFPLRLLSAAPSQTSVYFCASSYVGNTGELFFGEGSRLTVLEDLKNVFPPEVAVFEPSEAEISHTQKATLVCLATGFFPDHVELSWWVNGKEVHSGVSTDPQPLKEQPALNDSRYCLSSRLRVSATFWQNPRNHFRCQVQFYGLSENDEWTQDRAKPVTQIVSAEAWGRADCGFTSVSYQQGVLSATILYEILLGKATLYAVLVSALVLMAMVKRKDF

SEQ ID NO: 18 - DNA, 1812 bp, synthetic construct
  source 1..1812: mol_type = other DNA
atggagaccctcttgggcctgcttatcctttggctgcagctgcaatgggtgagcagcaaacaggaggtgacgcagattcctgcagctctgagtgtcccagaaggagaaaacttggttctcaactgcagtttcactgatagcgctatttacaacctccagtggtttaggcaggaccctgggaaaggtctcacatctctgttgcttattcagtcaagtcagagagagcaaacaagtggaagacttaatgcctcgctggataaatcatcaggacgtagtactttatacattgcagcttctcagcctggtgactcagccacctacctctgtgctgtgaggcccttatacggaggaagctacatacctacatttggaagaggaaccagccttattgttcatccgtacatccagaaccctgaccctgccgtgtaccagctgagagactctaaatccagtgacaagtctgtctgcctattcaccgattttgattctcaaacaaatgtgtcacaaagtaaggattctgatgtgtatatcacagacaaaactgtgctagacatgaggtctatggacttcaagagcaacagtgctgtggcctggagcaacaaatctgactttgcatgtgcaaacgccttcaacaacagcattattccagaagacaccttcttccccagcccagaaagttcctgtgatgtcaagctggtcgagaaaagctttgaaacagatacgaacctaaactttcaaaacctgtcagtgattgggttccgaatcctcctcctgaaagtggccgggtttaatctgctcatgacgctgcggctgtggtccagccaatgtactaactacgctttgttgaaactcgctggcgatgttgaaagtaaccccggtcctatgagcatcggcctcctgtgctgtgcagccttgtctctcctgtgggcaggtccagtgaatgctggtgtcactcagaccccaaaattccaggtcctgaagacaggacagagcatgacactgcagtgtgcccaggatatgaaccatgaatacatgtcctggtatcgacaagacccaggcatggggctgaggctgattcattactcagttggtgctggtatcactgaccaaggagaagtccccaatggctacaatgtctccagatcaaccacagaggatttcccgctcaggctgctgtcggctgctccctcccagacatctgtgtacttctgtgccagcagttacgtcgggaacaccggggagctgttttttggagaaggctctaggctgaccgtactggaggacctgaagaacgtgttcccacccgaggtcgctgtgtttgagccatcagaagcagagatctcccacacccaaaaggccacactggtgtgcctggccacaggcttcttccctgaccacgtggagctgagctggtgggtgaatgggaaggaggtgcacagtggggtcagcacggacccgcagcccctcaaggagcagcccgccctcaatgactccagatactgcctgagcagccgcctgagggtctcggccaccttctggcagaacccccgcaaccacttccgctgtcaagtccagttctacgggctctcggagaatgacgagtggacccaggatagggccaaacccgtcacccagatcgtcagcgccgaggcctggggtagagcagactgtggctttacctcggtgtcctaccagcaaggggtcctgtctgccaccatcctctatgagatcctgctagggaaggccaccctgtatgctgtgctggtcagcgcccttgtgttgatggccatggtcaagagaaaggatttctaa

SEQ ID NO: 19 - protein, 488 aa, synthetic construct
MGWSCIILFLVATATGVHSAIQLTQSPSSLSASVGDRVTITCRASQGISSALAWYQQKPGKAPKLLIYDASSLESGVPSRFSGSGSGTDFTLTISSLQPEDFATYYCQQFNSYPYTFGQGTKLEIKGGGGSGGGGSGGGGSEVQLVQSGAEVKKPGESLKISCKGSGYSFSSSWIGWVRQMPGKGLEWMGIIYPDDSDTRYSPSFQGQVTISADKSIRTAYLQWSSLKASDTAMYYCARHVTMIWGVIIDFWGQGTLVTVSSAAATTTPAPRPPTPAPTIASQPLSLRPEACRPAAGGAVHTRGLDFACDIYIWAPLAGTCGVLLLSLVITLYCKRGRKKLLYIFKQPFMRPVQTTQEEDGCSCRFPEEEEGGCELRVKFSRSADAPAYKQGQNQLYNELNLGRREEYDVLDKRRGRDPEMGGKPRRKNPQEGLYNELQKDKMAEAYSEIGMKGERRRGKGHDGLYQGLSTATKDTYDALHMQALPPR

SEQ ID NO: 20 - DNA, 1467 bp, synthetic construct
  source 1..1467: mol_type = other DNA
atgggctggtcttgcatcatcctgttcctcgtggccaccgccaccggcgtccacagcgccatccagctcacccagagcccctcgagcttgagtgcctcggtgggagaccgggtcactatcacctgccgagccagtcagggcatctcctccgcccttgcctggtaccagcagaagcccgggaaggcccccaagctgctgatctacgacgctagtagtctggagagtggcgtgccttcgcgcttctcgggcagtgggagtggcaccgacttcaccttgaccatctccagtctacagccggaagatttcgcgacctactactgtcagcaattcaactcttatccatacactttcggccaggggacaaagctggagatcaagggcgggggcgggagtggcggcggagggtccggaggcgggggctccgaggtgcaactagtccagagcggagccgaggtgaagaagcccggggagagtctaaagatctcttgcaagggctccggttactccttctcgagttcctggatcgggtgggtgcgacagatgccgggcaagggcctggagtggatgggcattatctaccccgacgactccgatacccgttatagtccatcgttccagggacaggtgaccatttccgccgacaagtctatcagaaccgcctatctgcagtggtccagtctgaaggcctctgacactgccatgtattattgcgccaggcacgttacgatgatctggggggtgatcatcgacttctggggccagggcacactcgtaaccgtcagttctgcggccgcaaccacgacgccagcgccgcgaccaccaacaccggcgcccaccatcgcgtcgcagcccctgtccctgcgcccagaggcgtgccggccagcggcggggggcgcagtgcacacgagggggctggacttcgcctgtgatatctacatctgggcgcccttggccgggacttgtggggtccttctcctgtcactggttatcaccctttactgcaaacggggcagaaagaaactcctgtatatattcaaacaaccatttatgagaccagtacaaactactcaagaggaagatggctgtagctgccgatttccagaagaagaagaaggaggatgtgaactgagagtgaagttcagcaggagcgcagacgcccccgcgtacaagcagggccagaaccagctctataacgagctcaatctaggacgaagagaggagtacgacgttttggacaagagacgtggccgggaccctgagatggggggaaagccgagaaggaagaaccctcaggaaggcctgtacaatgaactgcagaaagataagatggcggaggcctacagtgagattgggatgaaaggcgagcgccggaggggcaaggggcacgatggcctttaccagggtctcagtacagccaccaaggacacctacgacgcccttcacatgcaggccctgccccctcgctaa

SEQ ID NO: 21 - protein, 18 aa, Thosea asigna virus
EGRGSLLTCGDVEENPGP

SEQ ID NO: 22 - DNA, 54 bp, Artificial sequence
  source 1..54: mol_type = other DNA
gagggcagaggaagtcttctaacatgcggtgacgtggaggagaatcccggccct